European Patent Application EP 4 269 588 A1, published November 1, 2023. Title: An anti-EphA4 antibody. Applicant: EISAI R&D MANAGEMENT CO., LTD. The sequence listing filed with the application follows.

SEQUENCE LISTING (61 sequences)

SEQ ID NO: 1 - protein, 986 aa, Homo sapiens
MAGIFYFALFSCLFGICDAVTGSRVYPANEVTLLDSRSVQGELGWIASPLEGGWEEVSIMDEKNTPIRTYQVCNVMEPSQNNWLRTDWITREGAQRVYIEIKFTLRDCNSLPGVMGTCKETFNLYYYESDNDKERFIRENQFVKIDTIAADESFTQVDIGDRIMKLNTEIRDVGPLSKKGFYLAFQDVGACIALVSVRVFYKKCPLTVRNLAQFPDTITGADTSSLVEVRGSCVNNSEEKDVPKMYCGADGEWLVPIGNCLCNAGHEERSGECQACKIGYYKALSTDATCAKCPPHSYSVWEGATSCTCDRGFFRADNDAASMPCTRPPSAPLNLISNVNETSVNLEWSSPQNTGGRQDISYNVVCKKCGAGDPSKCRPCGSGVHYTPQQNGLKTTKVSITDLLAHTNYTFEIWAVNGVSKYNPNPDQSVSVTVTTNQAAPSSIALVQAKEVTRYSVALAWLEPDRPNGVILEYEVKYYEKDQNERSYRIVRTAARNTDIKGLNPLTSYVFHVRARTAAGYGDFSEPLEVTTNTVPSRIIGDGANSTVLLVSVSGSVVLVVILIAAFVISRRRSKYSKAKQEADEEKHLNQGVRTYVDPFTYEDPNQAVREFAKEIDASCIKIEKVIGVGEFGEVCSGRLKVPGKREICVAIKTLKAGYTDKQRRDFLSEASIMGQFDHPNIIHLEGVVTKCKPVMIITEYMENGSLDAFLRKNDGRFTVIQLVGMLRGIGSGMKYLSDMSYVHRDLAARNILVNSNLVCKVSDFGMSRVLEDDPEAAYTTRGGKIPIRWTAPEAIAYRKFTSASDVWSYGIVMWEVMSYGERPYWDMSNQDVIKAIEEGYRLPPPMDCPIALHQLMLDCWQKERSDRPKFGQIVNMLDKLIRNPNSLKRTGTESSRPNTALLDPSSPEFSAVVSVGDWLQAIKMDRYKDNFTAAGYTTLEAVVHVNQEDLARIGITAITHQNKILSSVQAMRTQMQQMHGRMVPV

SEQ ID NO: 2 - protein, 528 aa, Homo sapiens
VTGSRVYPANEVTLLDSRSVQGELGWIASPLEGGWEEVSIMDEKNTPIRTYQVCNVMEPSQNNWLRTDWITREGAQRVYIEIKFTLRDCNSLPGVMGTCKETFNLYYYESDNDKERFIRENQFVKIDTIAADESFTQVDIGDRIMKLNTEIRDVGPLSKKGFYLAFQDVGACIALVSVRVFYKKCPLTVRNLAQFPDTITGADTSSLVEVRGSCVNNSEEKDVPKMYCGADGEWLVPIGNCLCNAGHEERSGECQACKIGYYKALSTDATCAKCPPHSYSVWEGATSCTCDRGFFRADNDAASMPCTRPPSAPLNLISNVNETSVNLEWSSPQNTGGRQDISYNVVCKKCGAGDPSKCRPCGSGVHYTPQQNGLKTTKVSITDLLAHTNYTFEIWAVNGVSKYNPNPDQSVSVTVTTNQAAPSSIALVQAKEVTRYSVALAWLEPDRPNGVILEYEVKYYEKDQNERSYRIVRTAARNTDIKGLNPLTSYVFHVRARTAAGYGDFSEPLEVTTNTVPSRIIGDGANST

SEQ ID NO: 3 - protein, 1030 aa, Artificial Sequence
  Synthetic polypeptide
VTGSRVYPANEVTLLDSRSVQGELGWIASPLEGGWEEVSIMDEKNTPIRTYQVCNVMEPSQNNWLRTDWITREGAQRVYIEIKFTLRDCNSLPGVMGTCKETFNLYYYESDNDKERFIRENQFVKIDTIAADESFTQVDIGDRIMKLNTEIRDVGPLSKKGFYLAFQDVGACIALVSVRVFYKKCPLTVRNLAQFPDTITGADTSSLVEVRGSCVNNSEEKDVPKMYCGADGEWLVPIGNCLCNAGHEERSGECQACKIGYYKALSTDATCAKCPPHSYSVWEGATSCTCDRGFFRADNDAASMPCTRPPSAPLNLISNVNETSVNLEWSSPQNTGGRQDISYNVVCKKCGAGDPSKCRPCGSGVHYTPQQNGLKTTKVSITDLLAHTNYTFEIWAVNGVSKYNPNPDQSVSVTVTTNQAAPSSIALVQAKEVTRYSVALAWLEPDRPNGVILEYEVKYYEKDQNERSYRIVRTAARNTDIKGLNPLTSYVFHVRARTAAGYGDFSEPLEVTTNTVPSRIIGDGANSTAAAIIPVEEENPDFWNREAAEALGAAKKLQPAQTAAKNLIIFLGDGMGVSTVTAARILKGQKKDKLGPEIPLAMDRFPYVALSKTYNVDKHVPDSGATATAYLCGVKGNFQTIGLSAAARFNQCNTTRGNEVISVMNRAKKAGKSVGVVTTTRVQHASPAGTYAHTVNRNWYSDADVPASARQEGCQDIATQLISNMDIDVILGGGRKYMFRMGTPDPEYPDDYSQGGTRLDGKNLVQEWLAKRQGARYVWNRTELMQASLDPSVTHLMGLFEPGDMKYEIHRDSTLDPSLMEMTEAALRLLSRNPRGFFLFVEGGRIDHGHHESRAYRALTETIMFDDAIERAGQLTSEEDTLSLVTADHSHVFSFGGYPLRGSSIFGLAPGKARDRKAYTVLLYGNGPGYVLKDGARPDVTESESGSPEYRQQSAVPLDEETHAGEDVAVFARGPQAHLVHGVQEQTFIAHVMAFAACLEPYTACDLAPPAGTTDAAHPGHHHHHHHHHH

SEQ ID NO: 4 - protein, 772 aa, Artificial Sequence
  Synthetic polypeptide
VTGSRVYPANEVTLLDSRSVQGELGWIASPLEGGWEEVSIMDEKNTPIRTYQVCNVMEPSQNNWLRTDWITREGAQRVYIEIKFTLRDCNSLPGVMGTCKETFNLYYYESDNDKERFIRENQFVKIDTIAADESFTQVDIGDRIMKLNTEIRDVGPLSKKGFYLAFQDVGACIALVSVRVFYKKCPLTVRNLAQFPDTITGADTSSLVEVRGSCVNNSEEKDVPKMYCGADGEWLVPIGNCLCNAGHEERSGECQACKIGYYKALSTDATCAKCPPHSYSVWEGATSCTCDRGFFRADNDAASMPCTRPPSAPLNLISNVNETSVNLEWSSPQNTGGRQDISYNVVCKKCGAGDPSKCRPCGSGVHYTPQQNGLKTTKVSITDLLAHTNYTFEIWAVNGVSKYNPNPDQSVSVTVTTNQAAPSSIALVQAKEVTRYSVALAWLEPDRPNGVILEYEVKYYEKDQNERSYRIVRTAARNTDIKGLNPLTSYVFHVRARTAAGYGDFSEPLEVTTNTVPSRIIGDGANSTAAAPKSCDKTHTCPPCPAPELLGGPSVFLFPPKPKDTLMISRTPEVTCVVVDVSHEDPEVKFNWYVDGVEVHNAKTKPREEQYNSTYRVVSVLTVLHQDWLNGKEYKCKVSNKALPAPIEKTISKAKGQPREPQVYTLPPSREEMTKNQVSLTCLVKGFYPSDIAVEWESNGQPENNYKTTPPVLDSDGSFFLYSKLTVDKSRWQQGNVFSCSVMHEALHNHYTQKSLSLSPGKHHHHHHHHHH

SEQ ID NO: 5 - protein, 905 aa, Artificial Sequence
  Synthetic polypeptide
VTGSRVYPANEVTLLDSRSVQGELGWIASPLEGGWEEVSIMDEKNTPIRTYQVCNVMEPSQNNWLRTDWITREGAQRVYIEIKFTLRDCNSLPGVMGTCKETFNLYYYESDNDKERFIRENQFVKIDTIAADESFTQVDIGDRIMKLNTEIRDVGPLSKKGFYLAFQDVGACIALVSVRVFYKKCPLTVRNLAQFPDTITGADTSSLVEVRGSCVNNSEEKDVPKMYCGADGEWLVPIGNCLCNAGHEERSGECQACKIGYYKALSTDATCAKCPPHSYSVWEGATSCTCDRGFFRADNDAASMPCTRPPSAPLNLISNVNETSVNLEWSSPQNTGGRQDISYNVVCKKCGAGDPSKCRPCGSGVHYTPQQNGLKTTKVSITDLLAHTNYTFEIWAVNGVSKYNPNPDQSVSVTVTTNQAAPSSIALVQAKEVTRYSVALAWLEPDRPNGVILEYEVKYYEKDQNERSYRIVRTAARNTDIKGLNPLTSYVFHVRARTAAGYGDFSEPLEVTTNTVPSRIIGDGANSTAAAEEGKLVIWINGDKGYNGLAEVGKKFEKDTGIKVTVEHPDKLEEKFPQVAATGDGPDIIFWAHDRFGGYAQSGLLAEITPDKAFQDKLYPFTWDAVRYNGKLIAYPIAVEALSLIYNKDLLPNPPKTWEEIPALDKELKAKGKSALMFNLQEPYFTWPLIAADGGYAFKYENGKYDIKDVGVDNAGAKAGLTFLVDLIKNKHMNADTDYSIAEAAFNKGETAMTINGPWAWSNIDTSKVNYGVTVLPTFKGQPSKPFVGVLSAGINAASPNKELAKEFLENYLLTDEGLEAVNKDKPLGAVALKSYEEELAKDPRIAATMENAQKGEIMPNIPQMSAFWYAVRTAVINAASGRQTVDEALKDAQTHHHHHHHHHH

SEQ ID NO: 6 - protein, 19 aa, Artificial Sequence
  Synthetic polypeptide
MAGIFYFALFSCLFGICDA

SEQ ID NO: 7 - protein, 123 aa, Artificial Sequence
  Synthetic polypeptide
EVQLLESGGGLVQPGGSLRLSCAASGFTFSSYAMSWVRQAPGKGLEWVSAISGSGGSTYYADSVKGRFTISRDNSKNTLYLQMNSLRAEDTAVYYCARDSYYYWWLYYYFDYWGQGTLVTVSS

SEQ ID NO: 8 - protein, 108 aa, Artificial Sequence
  Synthetic polypeptide
SSELTQDPAVSVALGQTVRITCQGDSLRSYYASWYQQKPGQAPVLVIYGKNNRPSGIPDRFSGSSSGNTASLTITGAQAEDEADYYCQSSYSSSYSYVFGGGTKLTVL

SEQ ID NO: 9 - DNA, 369 bp, Artificial Sequence
  Synthetic oligonucleotide
gaagtgcagctgctggagagcgggggaggcctggtgcagcctggcggctctctgaggctgtcctgtgctgcctccggcttcacattttccagctacgctatgtcttgggtgcggcaggctccaggcaagggactggagtgggtgtctgctatctctggaagcggcggctccacctactatgctgacagcgtgaagggcaggttcacaatctctcgggataactccaagaataccctgtacctgcagatgaactccctgagggctgaggacacagccgtgtactattgtgctcgggatagctactattactggtggctgtattactatttcgactattggggccagggcacactggtgaccgtgtcttcc

SEQ ID NO: 10 - DNA, 324 bp, Artificial Sequence
  Synthetic oligonucleotide
tcttctgaactgacccaggaccccgctgtgtctgtggccctgggccagacagtgagaatcacctgccagggcgacagcctgcgctcttactatgcctcctggtaccagcagaagccaggccaggctcccgtgctggtcatctacggcaagaacaataggccttctggcatcccagatcggttttccggctccagctctggcaacacagccagcctgacaattacaggagctcaggctgaggatgaggctgattactattgccagtccagctactcttccagctactcctacgtgttcgggggagggacaaagctgaccgtgctg

SEQ ID NO: 11 - protein, 124 aa, Artificial Sequence
  Synthetic polypeptide
EVQLLESGGGLVQPGGSLRLSCAASGFTFSSFAMSWVRQAPGKGLEWVSAISGSGGSTYYADSVKGRFTISRDNSKNTLYLQMNSLRAEDTAVYYCARDDYYPYWWYYYYFDYWGQGTLVTVSS

SEQ ID NO: 12 - protein, 108 aa, Artificial Sequence
  Synthetic polypeptide
SSELTQDPAVSVALGQTVRITCQGDSLRSYFASWYQQKPGQAPVLVIYGKNNRPSGIPDRFSGSSSGNTASLTITGAQAEDEADYYCQSSYSSSYSYVFGGGTKLTVL

SEQ ID NO: 13 - DNA, 372 bp, Artificial Sequence
  Synthetic oligonucleotide
gaagtgcagctgctggagtccggtgggggcctggtgcagcccggcggctctctgagactgtcctgtgctgcctccggcttcaccttttccagcttcgctatgtcttgggtgcggcaggctcctggcaagggactggagtgggtgtctgctatcagcggctctggcggctccacatactatgccgacagcgtgaagggcaggtttaccatctctcgggataactccaagaatacactgtacctgcagatgaactctctgagggctgaggacaccgccgtgtactattgcgctcgggacgattactatccatactggtggtactattactatttcgattattggggccagggcaccctggtgacagtgtcttcc

SEQ ID NO: 14 - DNA, 324 bp, Artificial Sequence
  Synthetic oligonucleotide
tcttccgaactgacccaggaccccgctgtgtctgtggccctgggccagacagtgagaatcacctgccagggcgacagcctgcgctcttactttgcctcctggtatcagcagaagccaggccaggctcccgtgctggtcatctacggcaagaacaataggccttctggcatcccagatcggttctccggctccagctctggcaacacagccagcctgacaattacaggagctcaggctgaggatgaggctgattactattgccagtccagctattcttccagctactcctacgtgttcgggggagggacaaagctgaccgtgctg

SEQ ID NO: 15 - protein, 326 aa, Artificial Sequence
  Synthetic polypeptide
ASTKGPSVFPLAPSSRSTSESTAALGCLVKDYFPEPVTVSWNSGALTSGVHTFPAVLQSSGLYSLSSVVTVPSSNFGTQTYTCNVDHKPSNTKVDKTVERKSCVECPPCPAPPAAAPSVFLFPPKPKDTLMISRTPEVTCVVVDVSHEDPEVQFNWYVDGVEVHNAKTKPREEQFNSTFRVVSVLTVVHQDWLNGKEYKCKVSNKGLPAPIEKTISKTKGQPREPQVYTLPPSREEMTKNQVSLTCLVKGFYPSDIAVEWESNGQPENNYKTTPPMLDSDGSFFLYSKLTVDKSRWQQGNVFSCSVMHEALHNHYTQKSLSLSPGK

SEQ ID NO: 16 - protein, 329 aa, Artificial Sequence
  Synthetic polypeptide
ASTKGPSVFPLAPSSKSTSGGTAALGCLVKDYFPEPVTVSWNSGALTSGVHTFPAVLQSSGLYSLSSVVTVPSSSLGTQTYICNVNHKPSNTKVDKRVEPKSCDKTHTCPPCPAPPAAAPSVFLFPPKPKDTLMISRTPEVTCVVVDVSHEDPEVQFNWYVDGVEVHNAKTKPREEQFNSTFRVVSVLTVVHQDWLNGKEYKCKVSNKGLPAPIEKTISKTKGQPREPQVYTLPPSREEMTKNQVSLTCLVKGFYPSDIAVEWESNGQPENNYKTTPPMLDSDGSFFLYSKLTVDKSRWQQGNVFSCSVMHEALHNHYTQKSLSLSPGK

SEQ ID NO: 17 - protein, 106 aa, Artificial Sequence
  Synthetic polypeptide
GQPKAAPSVTLFPPSSEELQANKATLVCLISDFYPGAVTVAWKADSSPVKAGVETTTPSKQSNNKYAASSYLSLTPEQWKSHRSYSCQVTHEGSTVEKTVAPTECS

SEQ ID NO: 18 - DNA, 978 bp, Artificial Sequence
  Synthetic oligonucleotide
gcctccaccaagggaccatccgtgttcccactggccccaagctctaggtctacatccgagtctacagccgctctgggatgcctggtgaaggattacttccctgagccagtgacagtgagctggaactctggcgctctgacatctggcgtgcacacctttcctgccgtgctgcagtccagcggcctgtactccctgtcttccgtggtgaccgtgcccagctctaatttcggcacccagacatatacctgtaacgtggaccataagcctagcaatacaaaggtggataagaccgtggagagaaagtcttgcgtggagtgtcccccttgccctgccccacccgccgctgccccttccgtgttcctgtttcctccaaagccaaaggacacactgatgatctctcgcacacctgaggtgacctgcgtggtggtggacgtgagccacgaggatccagaggtgcagtttaactggtacgtggatggcgtggaggtgcataatgctaagaccaagcccagagaggagcagttcaactctacatttcgcgtggtgtccgtgctgaccgtggtgcaccaggactggctgaacggcaaggagtataagtgtaaggtgtctaataagggcctgcccgcccctatcgagaagacaatctccaagaccaagggccagcctagagagccacaggtgtacaccctgcccccttctcgcgaggagatgacaaagaaccaggtgtccctgacctgcctggtgaagggcttctatccttccgacatcgctgtggagtgggagagcaatggccagccagagaacaattacaagaccacaccacccatgctggactccgatggcagcttctttctgtatagcaagctgaccgtggataagtctcggtggcagcagggcaacgtgttctcctgctccgtgatgcacgaagccctgcacaatcattacacccagaaatccctgtccctgtcccccggcaaa

SEQ ID NO: 19 - DNA, 318 bp, Artificial Sequence
  Synthetic oligonucleotide
ggacagccaaaggctgctccttctgtgaccctgtttcccccttcttccgaggagctgcaggccaataaggccaccctggtgtgcctgatctctgacttctatccaggagctgtgacagtggcttggaaggctgatagctctccagtgaaggctggcgtggagaccacaaccccctccaagcagagcaacaataagtacgccgcttccagctatctgagcctgacaccagagcagtggaagtctcacaggtcttactcctgccaggtgacccacgaaggtagcacagtcgaaaaaaccgtcgctcccacagagtgttct

SEQ ID NO: 20 - protein, 449 aa, Artificial Sequence
  Synthetic polypeptide
EVQLLESGGGLVQPGGSLRLSCAASGFTFSSYAMSWVRQAPGKGLEWVSAISGSGGSTYYADSVKGRFTISRDNSKNTLYLQMNSLRAEDTAVYYCARDSYYYWWLYYYFDYWGQGTLVTVSSASTKGPSVFPLAPSSRSTSESTAALGCLVKDYFPEPVTVSWNSGALTSGVHTFPAVLQSSGLYSLSSVVTVPSSNFGTQTYTCNVDHKPSNTKVDKTVERKSCVECPPCPAPPAAAPSVFLFPPKPKDTLMISRTPEVTCVVVDVSHEDPEVQFNWYVDGVEVHNAKTKPREEQFNSTFRVVSVLTVVHQDWLNGKEYKCKVSNKGLPAPIEKTISKTKGQPREPQVYTLPPSREEMTKNQVSLTCLVKGFYPSDIAVEWESNGQPENNYKTTPPMLDSDGSFFLYSKLTVDKSRWQQGNVFSCSVMHEALHNHYTQKSLSLSPGK

SEQ ID NO: 21 - protein, 214 aa, Artificial Sequence
  Synthetic polypeptide
SSELTQDPAVSVALGQTVRITCQGDSLRSYYASWYQQKPGQAPVLVIYGKNNRPSGIPDRFSGSSSGNTASLTITGAQAEDEADYYCQSSYSSSYSYVFGGGTKLTVLGQPKAAPSVTLFPPSSEELQANKATLVCLISDFYPGAVTVAWKADSSPVKAGVETTTPSKQSNNKYAASSYLSLTPEQWKSHRSYSCQVTHEGSTVEKTVAPTECS

SEQ ID NO: 22 - DNA, 1347 bp, Artificial Sequence
  Synthetic oligonucleotide
gaagtgcagctgctggagagcgggggaggcctggtgcagcctggcggctctctgaggctgtcctgtgctgcctccggcttcacattttccagctacgctatgtcttgggtgcggcaggctccaggcaagggactggagtgggtgtctgctatctctggaagcggcggctccacctactatgctgacagcgtgaagggcaggttcacaatctctcgggataactccaagaataccctgtacctgcagatgaactccctgagggctgaggacacagccgtgtactattgtgctcgggatagctactattactggtggctgtattactatttcgactattggggccagggcacactggtgaccgtgtcttccgcctccaccaagggaccatccgtgttcccactggccccaagctctaggtctacatccgagtctacagccgctctgggatgcctggtgaaggattacttccctgagccagtgacagtgagctggaactctggcgctctgacatctggcgtgcacacctttcctgccgtgctgcagtccagcggcctgtactccctgtcttccgtggtgaccgtgcccagctctaatttcggcacccagacatatacctgtaacgtggaccataagcctagcaatacaaaggtggataagaccgtggagagaaagtcttgcgtggagtgtcccccttgccctgccccacccgccgctgccccttccgtgttcctgtttcctccaaagccaaaggacacactgatgatctctcgcacacctgaggtgacctgcgtggtggtggacgtgagccacgaggatccagaggtgcagtttaactggtacgtggatggcgtggaggtgcataatgctaagaccaagcccagagaggagcagttcaactctacatttcgcgtggtgtccgtgctgaccgtggtgcaccaggactggctgaacggcaaggagtataagtgtaaggtgtctaataagggcctgcccgcccctatcgagaagacaatctccaagaccaagggccagcctagagagccacaggtgtacaccctgcccccttctcgcgaggagatgacaaagaaccaggtgtccctgacctgcctggtgaagggcttctatccttccgacatcgctgtggagtgggagagcaatggccagccagagaacaattacaagaccacaccacccatgctggactccgatggcagcttctttctgtatagcaagctgaccgtggataagtctcggtggcagcagggcaacgtgttctcctgctccgtgatgcacgaagccctgcacaatcattacacccagaaatccctgtccctgtcccccggcaaa

SEQ ID NO: 23 - DNA, 642 bp, Artificial Sequence
  Synthetic oligonucleotide
tcttctgaactgacccaggaccccgctgtgtctgtggccctgggccagacagtgagaatcacctgccagggcgacagcctgcgctcttactatgcctcctggtaccagcagaagccaggccaggctcccgtgctggtcatctacggcaagaacaataggccttctggcatcccagatcggttttccggctccagctctggcaacacagccagcctgacaattacaggagctcaggctgaggatgaggctgattactattgccagtccagctactcttccagctactcctacgtgttcgggggagggacaaagctgaccgtgctgggacagccaaaggctgctccttctgtgaccctgtttcccccttcttccgaggagctgcaggccaataaggccaccctggtgtgcctgatctctgacttctatccaggagctgtgacagtggcttggaaggctgatagctctccagtgaaggctggcgtggagaccacaaccccctccaagcagagcaacaataagtacgccgcttccagctatctgagcctgacaccagagcagtggaagtctcacaggtcttactcctgccaggtgacccacgaaggtagcacagtcgaaaaaaccgtcgctcccacagagtgttct

SEQ ID NO: 24 - DNA, 987 bp, Artificial Sequence
  Synthetic oligonucleotide
gcctccaccaagggaccttccgtgttcccactggccccaagctctaagtccaccagcggcggcacagccgctctgggctgtctggtgaaggactacttccctgagccagtgacagtgagctggaactctggcgctctgacctccggcgtgcacacatttccagccgtgctgcagtccagcggcctgtacagcctgtcttccgtggtgaccgtgcccagctcttccctgggcacccagacatatatctgcaacgtgaatcacaagcctagcaatacaaaggtggacaagagagtggagccaaagtcttgtgataagacccatacatgccctccatgtcctgccccacccgccgctgccccttccgtgttcctgtttcctccaaagccaaaggacaccctgatgatctctcgcacccctgaggtgacatgcgtggtggtggacgtgagccacgaggatcctgaggtgcagttcaactggtacgtggatggcgtggaggtgcataatgctaagacaaagccaagagaggagcagttcaactctacctttcgcgtggtgtccgtgctgacagtggtgcatcaggattggctgaacggcaaggagtataagtgcaaggtgtctaataagggcctgcccgcccctatcgagaagaccatctccaagacaaagggccagcctagagagccacaggtgtacaccctgcccccttctcgcgaggagatgaccaagaaccaggtgtccctgacatgtctggtgaagggcttctatccctccgacatcgctgtggagtgggagagcaatggccagcctgagaacaattacaagaccacaccacccatgctggactccgatggcagcttctttctgtatagcaagctgaccgtggataagtctaggtggcagcagggcaacgtgttctcctgttccgtgatgcacgaagccctgcacaatcattacacccagaaaagcctgagcctgtcccccggaaaa

SEQ ID NO: 25 - DNA, 318 bp, Artificial Sequence
  Synthetic oligonucleotide
ggacagccaaaggctgctccttctgtgaccctgtttcccccttcttccgaggagctgcaggccaataaggccaccctggtgtgcctgatctctgacttctacccaggagctgtgacagtggcttggaaggctgatagctctccagtgaaggctggcgtggagaccacaaccccctccaagcagagcaacaataagtacgccgcttccagctatctgagcctgacaccagagcagtggaagtctcacaggtcttattcctgccaggtgacccacgaaggttccacagtcgaaaagaccgtcgctcctaccgagtgctcc

SEQ ID NO: 26 - protein, 453 aa, Artificial Sequence
  Synthetic polypeptide
EVQLLESGGGLVQPGGSLRLSCAASGFTFSSFAMSWVRQAPGKGLEWVSAISGSGGSTYYADSVKGRFTISRDNSKNTLYLQMNSLRAEDTAVYYCARDDYYPYWWYYYYFDYWGQGTLVTVSSASTKGPSVFPLAPSSKSTSGGTAALGCLVKDYFPEPVTVSWNSGALTSGVHTFPAVLQSSGLYSLSSVVTVPSSSLGTQTYICNVNHKPSNTKVDKRVEPKSCDKTHTCPPCPAPPAAAPSVFLFPPKPKDTLMISRTPEVTCVVVDVSHEDPEVQFNWYVDGVEVHNAKTKPREEQFNSTFRVVSVLTVVHQDWLNGKEYKCKVSNKGLPAPIEKTISKTKGQPREPQVYTLPPSREEMTKNQVSLTCLVKGFYPSDIAVEWESNGQPENNYKTTPPMLDSDGSFFLYSKLTVDKSRWQQGNVFSCSVMHEALHNHYTQKSLSLSPGK

SEQ ID NO: 27 - protein, 214 aa, Artificial Sequence
  Synthetic polypeptide
SSELTQDPAVSVALGQTVRITCQGDSLRSYFASWYQQKPGQAPVLVIYGKNNRPSGIPDRFSGSSSGNTASLTITGAQAEDEADYYCQSSYSSSYSYVFGGGTKLTVLGQPKAAPSVTLFPPSSEELQANKATLVCLISDFYPGAVTVAWKADSSPVKAGVETTTPSKQSNNKYAASSYLSLTPEQWKSHRSYSCQVTHEGSTVEKTVAPTECS

SEQ ID NO: 28 - DNA, 1359 bp, Artificial Sequence
  Synthetic oligonucleotide
gaagtgcagctgctggagtccggtgggggcctggtgcagcccggcggctctctgagactgtcctgtgctgcctccggcttcaccttttccagcttcgctatgtcttgggtgcggcaggctcctggcaagggactggagtgggtgtctgctatcagcggctctggcggctccacatactatgccgacagcgtgaagggcaggtttaccatctctcgggataactccaagaatacactgtacctgcagatgaactctctgagggctgaggacaccgccgtgtactattgcgctcgggacgattactatccatactggtggtactattactatttcgattattggggccagggcaccctggtgacagtgtcttccgcctccaccaagggaccttccgtgttcccactggccccaagctctaagtccaccagcggcggcacagccgctctgggctgtctggtgaaggactacttccctgagccagtgacagtgagctggaactctggcgctctgacctccggcgtgcacacatttccagccgtgctgcagtccagcggcctgtacagcctgtcttccgtggtgaccgtgcccagctcttccctgggcacccagacatatatctgcaacgtgaatcacaagcctagcaatacaaaggtggacaagagagtggagccaaagtcttgtgataagacccatacatgccctccatgtcctgccccacccgccgctgccccttccgtgttcctgtttcctccaaagccaaaggacaccctgatgatctctcgcacccctgaggtgacatgcgtggtggtggacgtgagccacgaggatcctgaggtgcagttcaactggtacgtggatggcgtggaggtgcataatgctaagacaaagccaagagaggagcagttcaactctacctttcgcgtggtgtccgtgctgacagtggtgcatcaggattggctgaacggcaaggagtataagtgcaaggtgtctaataagggcctgcccgcccctatcgagaagaccatctccaagacaaagggccagcctagagagccacaggtgtacaccctgcccccttctcgcgaggagatgaccaagaaccaggtgtccctgacatgtctggtgaagggcttctatccctccgacatcgctgtggagtgggagagcaatggccagcctgagaacaattacaagaccacaccacccatgctggactccgatggcagcttctttctgtatagcaagctgaccgtggataagtctaggtggcagcagggcaacgtgttctcctgttccgtgatgcacgaagccctgcacaatcattacacccagaaaagcctgagcctgtcccccggaaaa

SEQ ID NO: 29 - DNA, 642 bp, Artificial Sequence
  Synthetic oligonucleotide
tcttccgaactgacccaggaccccgctgtgtctgtggccctgggccagacagtgagaatcacctgccagggcgacagcctgcgctcttactttgcctcctggtatcagcagaagccaggccaggctcccgtgctggtcatctacggcaagaacaataggccttctggcatcccagatcggttctccggctccagctctggcaacacagccagcctgacaattacaggagctcaggctgaggatgaggctgattactattgccagtccagctattcttccagctactcctacgtgttcgggggagggacaaagctgaccgtgctgggacagccaaaggctgctccttctgtgaccctgtttcccccttcttccgaggagctgcaggccaataaggccaccctggtgtgcctgatctctgacttctacccaggagctgtgacagtggcttggaaggctgatagctctccagtgaaggctggcgtggagaccacaaccccctccaagcagagcaacaataagtacgccgcttccagctatctgagcctgacaccagagcagtggaagtctcacaggtcttattcctgccaggtgacccacgaaggttccacagtcgaaaagaccgtcgctcctaccgagtgctcc

SEQ ID NO: 30 - protein, 5 aa, Artificial Sequence
  Synthetic polypeptide
SYAMS

SEQ ID NO: 31 - protein, 17 aa, Artificial Sequence
  Synthetic polypeptide
AISGSGGSTYYADSVKG

SEQ ID NO: 32 - protein, 14 aa, Artificial Sequence
  Synthetic polypeptide
DSYYYWWLYYYFDY

SEQ ID NO: 33 - protein, 11 aa, Artificial Sequence
  Synthetic polypeptide
QGDSLRSYYAS

SEQ ID NO: 34 - protein, 7 aa, Artificial Sequence
  Synthetic polypeptide
GKNNRPS

SEQ ID NO: 35 - protein, 11 aa, Artificial Sequence
  Synthetic polypeptide
QSSYSSSYSYV

SEQ ID NO: 36 - DNA, 15 bp, Artificial Sequence
  Synthetic oligonucleotide
agctacgctatgtct

SEQ ID NO: 37 - DNA, 51 bp, Artificial Sequence
  Synthetic oligonucleotide
gctatctctggaagcggcggctccacctactatgctgacagcgtgaagggc

SEQ ID NO: 38 - DNA, 42 bp, Artificial Sequence
  Synthetic oligonucleotide
gatagctactattactggtggctgtattactatttcgactat

SEQ ID NO: 39 - DNA, 33 bp, Artificial Sequence
  Synthetic oligonucleotide
cagggcgacagcctgcgctcttactatgcctcc

SEQ ID NO: 40 - DNA, 21 bp, Artificial Sequence
  Synthetic oligonucleotide
ggcaagaacaataggccttct

SEQ ID NO: 41 - DNA, 33 bp, Artificial Sequence
  Synthetic oligonucleotide
cagtccagctactcttccagctactcctacgtg

SEQ ID NO: 42 - protein, 5 aa, Artificial Sequence
  Synthetic polypeptide
SFAMS

SEQ ID NO: 43 - protein, 15 aa, Artificial Sequence
  Synthetic polypeptide
DDYYPYWWYYYYFDY

SEQ ID NO: 44 - protein, 11 aa, Artificial Sequence
  Synthetic polypeptide
QGDSLRSYFAS

SEQ ID NO: 45 - DNA, 15 bp, Artificial Sequence
  Synthetic oligonucleotide
agcttcgctatgtct

SEQ ID NO: 46 - DNA, 51 bp, Artificial Sequence
  Synthetic oligonucleotide
gctatcagcggctctggcggctccacatactatgccgacagcgtgaagggc

SEQ ID NO: 47 - DNA, 45 bp, Artificial Sequence
  Synthetic oligonucleotide
gacgattactatccatactggtggtactattactatttcgattat

SEQ ID NO: 48 - DNA, 33 bp, Artificial Sequence
  Synthetic oligonucleotide
cagggcgacagcctgcgctcttactttgcctcc

SEQ ID NO: 49 - DNA, 21 bp, Artificial Sequence
  Synthetic oligonucleotide
ggcaagaacaataggccttct

SEQ ID NO: 50 - DNA, 33 bp, Artificial Sequence
  Synthetic oligonucleotide
cagtccagctattcttccagctactcctacgtg

SEQ ID NO: 51 - protein, 986 aa, Macaca mulatta
MAGIFYFALFSCLFGICDAVTGSRVYPANEVTLLDSRSVQGELGWIASPLEGGWEEVSIMDEKNTPIRTYQVCNVMEPSQNNWLRTDWITREGAQRVYIEIKFTLRDCNSLPGVMGTCKETFNLYYYESDNDKERFIRENQFVKIDTIAADESFTQVDIGDRIMKLNTEIRDVGPLSKKGFYLAFQDVGACIALVSVRVFYKKCPLTVRNLAQFPDTITGADTSSLVEVRGSCVNNSEEKDVPKMYCGADGEWLVPIGNCLCNAGHEERSGECQACKIGYYKALSTDATCAKCPPHSYSVWEGATSCTCDRGFFRADNDAASMPCTRPPSAPLNLISNVNETSVNLEWSSPQNTGGRQDISYNVVCKKCGAGDPSKCRPCGSGVHYTPQQNGLKTTKVSITDLLAHTNYTFEIWAVNGVSKYNPSPDQSVSVTVTTNQAAPSSIALVQAKEVTRYSVALAWLEPDRPNGVILEYEVKYYEKDQNERSYRIVRTAARNTDIKGLNPLTSYVFHVRARTAAGYGDFSEPLEVTTNTVPSRIIGDGANSTVLLVSVSGSVVLVVILIAAFVISRRRSKYSKAKQEADEEKHLNQGVRTYVDPFTYEDPNQAVREFAKEIDASCIKIEKVIGVGEFGEVCSGRLKVPGKREICVAIKTLKAGYTDKQRRDFLSEASIMGQFDHPNIIHLEGVVTKCKPVMIITEYMENGSLDAFLRKNDGRFTVIQLVGMLRGIGSGMKYLSDMSYVHRDLAARNILVNSNLVCKVSDFGMSRVLEDDPEAAYTTRGGKIPIRWTAPEAIAYRKFTSASDVWSYGIVMWEVMSYGERPYWDMSNQDVIKAIEEGYRLPPPMDCPIALHQLMLDCWQKERSDRPKFGQIVNMLDKLIRNPNSLKRTGTESSRPNTALLDPSSPEFSAVVSVGDWLQAIKMDRYKDNFTAAGYTTLEAVVHVNQEDLARIGITAITHQNKILSSVQAMRTQMQQMHGRMVPV

SEQ ID NO: 52 - protein, 528 aa, Macaca mulatta
VTGSRVYPANEVTLLDSRSVQGELGWIASPLEGGWEEVSIMDEKNTPIRTYQVCNVMEPSQNNWLRTDWITREGAQRVYIEIKFTLRDCNSLPGVMGTCKETFNLYYYESDNDKERFIRENQFVKIDTIAADESFTQVDIGDRIMKLNTEIRDVGPLSKKGFYLAFQDVGACIALVSVRVFYKKCPLTVRNLAQFPDTITGADTSSLVEVRGSCVNNSEEKDVPKMYCGADGEWLVPIGNCLCNAGHEERSGECQACKIGYYKALSTDATCAKCPPHSYSVWEGATSCTCDRGFFRADNDAASMPCTRPPSAPLNLISNVNETSVNLEWSSPQNTGGRQDISYNVVCKKCGAGDPSKCRPCGSGVHYTPQQNGLKTTKVSITDLLAHTNYTFEIWAVNGVSKYNPSPDQSVSVTVTTNQAAPSSIALVQAKEVTRYSVALAWLEPDRPNGVILEYEVKYYEKDQNERSYRIVRTAARNTDIKGLNPLTSYVFHVRARTAAGYGDFSEPLEVTTNTVPSRIIGDGANST

SEQ ID NO: 53 - protein, 986 aa, Rattus norvegicus
MAGIFYFILFSFLFGICDAVTGSRVYPANEVTLLDSRSVQGELGWIASPLEGGWEEVSIMDEKNTPIRTYQVCNVMEASQNNWLRTDWITREGAQRVYIEIKFTLRDCNSLPGVMGTCKETFNLYYYESDNDKERFIRESQFGKIDTIAADESFTQVDIGDRIMKLNTEIRDVGPLSKKGFYLAFQDVGACIALVSVRVFYKKCPLTVRNLAQFPDTITGADTSSLVEVRGSCVNNSEEKDVPKMYCGADGEWLVPIGNCLCNAGHEEQNGECQACKIGYYKALSTDATCAKCPPHSYSVWEGATSCTCDRGFFRADNDAASMPCTRPPSAPLNLISNVNETSVNLEWSSPQNTGGRQDISYNVVCKKCGAGDPSKCRPCGSGVHYTPQQNGLKTTRVSITDLLAHTNYTFEIWAVNGVSKYNPSPDQSVSVTVTTNQAAPSSIALVQAKEVTRYSVALAWLEPDRPNGVILEYEVKYYEKDQNERSYRIVRTAARNTDIKGLNPLTSYVFHVRARTAAGYGDFSEPLEVTTNTVPSRIIGDGANSTVLLVSVSGSVVLVVILIAAFVISRRRSKYSQAKQEADEEKHLNQGVRTYVDPFTYEDPNQAVREFAKEIDASCIKIEKVIGVGEFGEVCSGRLKVPGKREICVAIKTLKAGYTDKQRRDFLSEASIMGQFDHPNIIHLEGVVTKCKPVMIITEYMENGSLDAFLRKNDGRFTVIQLVGMLRGIGSGMKYLSDMSYVHRDLAARNILVNSNLVCKVSDFGMSRVLEDDPEAAYTTRGGKIPIRWTAPEAIAYRKFTSASDVWSYGIVMWEVMSYGERPYWDMSNQDVIKAIEEGYRLPPPMDCPIALHQLMLDCWQKERSDRPKFGQIVNMLDKLIRNPNSLKRTGPESSRPNTALLDPSSPEFSAVVSVGDWLQAIKMDRYKDNFTAAGYTTLEAVVHMSQDDLARIGITAITHQNKILSSVQAMRTQMQQMHGRMVPV

SEQ ID NO: 54 - protein, 528 aa, Rattus norvegicus
VTGSRVYPANEVTLLDSRSVQGELGWIASPLEGGWEEVSIMDEKNTPIRTYQVCNVMEASQNNWLRTDWITREGAQRVYIEIKFTLRDCNSLPGVMGTCKETFNLYYYESDNDKERFIRESQFGKIDTIAADESFTQVDIGDRIMKLNTEIRDVGPLSKKGFYLAFQDVGACIALVSVRVFYKKCPLTVRNLAQFPDTITGADTSSLVEVRGSCVNNSEEKDVPKMYCGADGEWLVPIGNCLCNAGHEEQNGECQACKIGYYKALSTDATCAKCPPHSYSVWEGATSCTCDRGFFRADNDAASMPCTRPPSAPLNLISNVNETSVNLEWSSPQNTGGRQDISYNVVCKKCGAGDPSKCRPCGSGVHYTPQQNGLKTTRVSITDLLAHTNYTFEIWAVNGVSKYNPSPDQSVSVTVTTNQAAPSSIALVQAKEVTRYSVALAWLEPDRPNGVILEYEVKYYEKDQNERSYRIVRTAARNTDIKGLNPLTSYVFHVRARTAAGYGDFSEPLEVTTNTVPSRIIGDGANST

SEQ ID NO: 55 - protein, 986 aa, Mus musculus
MAGIFYFILFSFLFGICDAVTGSRVYPANEVTLLDSRSVQGELGWIASPLEGGWEEVSIMDEKNTPIRTYQVCNVMEASQNNWLRTDWITREGAQRVYIEIKFTLRDCNSLPGVMGTCKETFNLYYYESDNDKERFIRESQFGKIDTIAADESFTQVDIGDRIMKLNTEIRDVGPLSKKGFYLAFQDVGACIALVSVRVFYKKCPLTVRNLAQFPDTITGADTSSLVEVRGSCVNNSEEKDVPKMYCGADGEWLVPIGNCLCNAGHEEQNGECQACKIGYYKALSTDASCAKCPPHSYSVWEGATSCTCDRGFFRADNDAASMPCTRPPSAPLNLISNVNETSVNLEWSSPQNTGGRQDISYNVVCKKCGAGDPSKCRPCGSGVHYTPQQNGLKTTRVSITDLLAHTNYTFEIWAVNGVSKYNPSPDQSVSVTVTTNQAAPSSIALVQAKEVTRYSVALAWLEPDRPNGVILEYEVKYYEKDQNERSYRIVRTAARNTDIKGLNPLTSYVFHVRARTAAGYGDFSEPLEVTTNTVPSRIIGDGANSTVLLVSVSGSVVLVVILIAAFVISRRRSKYSKAKQEADEEKHLNQGVRTYVDPFTYEDPNQAVREFAKEIDASCIKIEKVIGVGEFGEVCSGRLKVPGKREICVAIKTLKAGYTDKQRRDFLSEASIMGQFDHPNIIHLEGVVTKCKPVMIITEYMENGSLDAFLRKNDGRFTVIQLVGMLRGIGSGMKYLSDMSYVHRDLAARNILVNSNLVCKVSDFGMSRVLEDDPEAAYTTRGGKIPIRWTAPEAIAYRKFTSASDVWSYGIVMWEVMSYGERPYWDMSNQDVIKAIEEGYRLPPPMDCPIALHQLMLDCWQKERSDRPKFGQIVNMLDKLIRNPNSLKRTGSESSRPNTALLDPSSPEFSAVVSVGDWLQAIKMDRYKDNFTAAGYTTLEAVVHMSQDDLARIGITAITHQNKILSSVQAMRTQMQQMHGRMVPV

SEQ ID NO: 56 - protein, 528 aa, Mus musculus
VTGSRVYPANEVTLLDSRSVQGELGWIASPLEGGWEEVSIMDEKNTPIRTYQVCNVMEASQNNWLRTDWITREGAQRVYIEIKFTLRDCNSLPGVMGTCKETFNLYYYESDNDKERFIRESQFGKIDTIAADESFTQVDIGDRIMKLNTEIRDVGPLSKKGFYLAFQDVGACIALVSVRVFYKKCPLTVRNLAQFPDTITGADTSSLVEVRGSCVNNSEEKDVPKMYCGADGEWLVPIGNCLCNAGHEEQNGECQACKIGYYKALSTDASCAKCPPHSYSVWEGATSCTCDRGFFRADNDAASMPCTRPPSAPLNLISNVNETSVNLEWSSPQNTGGRQDISYNVVCKKCGAGDPSKCRPCGSGVHYTPQQNGLKTTRVSITDLLAHTNYTFEIWAVNGVSKYNPSPDQSVSVTVTTNQAAPSSIALVQAKEVTRYSVALAWLEPDRPNGVILEYEVKYYEKDQNERSYRIVRTAARNTDIKGLNPLTSYVFHVRARTAAGYGDFSEPLEVTTNTVPSRIIGDGANST

SEQ ID NO: 57 - protein, 15 aa, Artificial Sequence
  Synthetic polypeptide
MSALLILALVGAAVA

SEQ ID NO: 58 - protein, 209 aa, Homo sapiens
MAGIFYFALFSCLFGICDAVTGSRVYPANEVTLLDSRSVQGELGWIASPLEGGWEEVSIMDEKNTPIRTYQVCNVMEPSQNNWLRTDWITREGAQRVYIEIKFTLRDCNSLPGVMGTCKETFNLYYYESDNDKERFIRENQFVKIDTIAADESFTQVDIGDRIMKLNTEIRDVGPLSKKGFYLAFQDVGACIALVSVRVFYKKCPLTVR

SEQ ID NO: 59 - protein, 114 aa, Homo sapiens
TRPPSAPLNLISNVNETSVNLEWSSPQNTGGRQDISYNVVCKKCGAGDPSKCRPCGSGVHYTPQQNGLKTTKVSITDLLAHTNYTFEIWAVNGVSKYNPNPDQSVSVTVTTNQA

SEQ ID NO: 60 - protein, 112 aa, Homo sapiens
TNQAAPSSIALVQAKEVTRYSVALAWLEPDRPNGVILEYEVKYYEKDQNERSYRIVRTAARNTDIKGLNPLTSYVFHVRARTAAGYGDFSEPLEVTTNTVPSRIIGDGANST

SEQ ID NO: 61 - protein, 374 aa, Artificial Sequence
  Synthetic polypeptide
EEGKLVIWINGDKGYNGLAEVGKKFEKDTGIKVTVEHPDKLEEKFPQVAATGDGPDIIFWAHDRFGGYAQSGLLAEITPDKAFQDKLYPFTWDAVRYNGKLIAYPIAVEALSLIYNKDLLPNPPKTWEEIPALDKELKAKGKSALMFNLQEPYFTWPLIAADGGYAFKYENGKYDIKDVGVDNAGAKAGLTFLVDLIKNKHMNADTDYSIAEAAFNKGETAMTINGPWAWSNIDTSKVNYGVTVLPTFKGQPSKPFVGVLSAGINAASPNKELAKEFLENYLLTDEGLEAVNKDKPLGAVALKSYEEELAKDPRIAATMENAQKGEIMPNIPQMSAFWYAVRTAVINAASGRQTVDEALKDAQTHHHHHHHHHH